European Patent Application EP 4 428 252 A1, published September 11, 2024. Title: Oligonucleotide primers for the identification of a bacterium of the genus Bacillus. Applicant: Kerry Group Services International Limited. Application EP. The sequence listing filed with the application follows.

SEQUENCE LISTING (6 sequences)

SEQ ID NO: 1 - DNA, 20 bp, synthetic construct
  source 1..20: mol_type = other DNA
accacttccccaacggtttt

SEQ ID NO: 2 - DNA, 19 bp, synthetic construct
  source 1..19: mol_type = other DNA
aacccctcaaaacagccaa

SEQ ID NO: 3 - DNA, 21 bp, synthetic construct
  source 1..21: mol_type = other DNA
tcgctgagcagagaatgaacc

SEQ ID NO: 4 - DNA, 20 bp, synthetic construct
  source 1..20: mol_type = other DNA
cggaagctcagggttctttt

SEQ ID NO: 5 - DNA, 21 bp, synthetic construct
  source 1..21: mol_type = other DNA
tgggttttcatccattagtcg

SEQ ID NO: 6 - DNA, 20 bp, synthetic construct
  source 1..20: mol_type = other DNA
aaggtgcggaagaaggatgg